European Patent Specification EP 3 641 834 B1, published October 4, 2023. Title: MESSENGER RNA THERAPY FOR THE TREATMENT OF FRIEDREICH'S ATAXIA. Applicant: TRANSLATE BIO, INC. The sequence listing filed with the application follows.

SEQUENCE LISTING (16 sequences)

SEQ ID NO: 1 - RNA, 633 nt, Artificial Sequence
  source: /note="Description of Artificial Sequence: Synthetic polynucleotide"
auguggacccugggucggagagcuguggccggucugcuggcuucccccucaccggcacaagcgcagacccugacuagagugccuaggcccgcugaacucgcaccacugugcggcagacggggacuccggacugacaucgaugccaccuguaccccgcgaagggcaucuagcaaucagcgcggacugaaccagaucuggaacgugaagaagcaguccguguaccugaugaaucugcgcaaauccggcacucucggacacccgggaucgcuggaugagacuacuuacgagcgcuuggccgaagaaacccuggauucgcuggccgaguuuuucgaggaccuggccgacaagcccuacacguucgaggacuacgacguguccuucggaucgggcgugcugaccgugaagcucggcggggauuuggggaccuacgugaucaacaagcagacaccgaacaagcaaauuuggcucuccuccccuuccuccggaccuaagcgcuacgacuggaccgggaagaacugggucuacucccaugacggcgucagccuucacgaacugcuggccgccgaacugacuaaggcccucaaaacuaagcuggaccugucgagccuugccuauuccggaaaggacgccuga

SEQ ID NO: 2 - RNA, 633 nt, Artificial Sequence
  source: /note="Description of Artificial Sequence: Synthetic polynucleotide"
auguggacccugggacgcagagccguggcuggccuucuggccuccccaagcccugcccaagcccagaccuugacuagagugccuagaccggccgaacucgcuccccugugcggacggaggggacucaggacugacaucgacgcaacaugcacuccaagacgcgccuccagcaaccagcggggccucaaccagauuuggaacgugaaaaagcaguccgucuaucugaugaaccuccgcaaguccggcaccuuggggcaucccgggucacuggaugaaaccaccuacgaacggcuggccgaagagacucucgacucccuggccgaguucuucgaggaccuggcggauaagccguacacuuucgaggacuacgaugucucuuucggauccggcgugcugaccgugaagcucgguggcgaccucggaacuuacgugaucaacaagcaaacgcccaacaagcagaucuggcuguccucgccgucaucgggaccuaagcgcuacgauuggaccgggaagaauuggguguacucgcacgacggugucagccugcacgagcugcuugcggcggaacugaccaaggcacucaagaccaaacuggaccuguccagccuggccuacuccggaaaggacgccuag

SEQ ID NO: 3 - RNA, 633 nt, Artificial Sequence
  source: /note="Description of Artificial Sequence: Synthetic polynucleotide"
auguggacucugggccggagagcuguggcaggccuucucgccucgccauccccugcccaagcgcagacccugacuagggucccuaggccugccgaguuggcaccguugugcggucggagaggacugcgcaccgacaucgaugccaccuguacuccucggagagccucguccaaccagcggggccugaaccagaucuggaacgugaagaaacaguccgucuaccugaugaaccuccgcaagucgggaacccugggacauccggguucccuggaugagacuacguacgaacggcuggcggaagaaacccuggacucccuggcggaguucuucgaggaccuggcugacaagcccuacacuuuugaggacuacgacgugucauucggaagcggaguguugacagugaagcuggggggcgaucugggaaccuacgugaucaacaagcagaccccgaacaagcaaauuuggcuguccucacccuccuccggaccuaaacgcuacgacuggaccgggaagaacuggguguauagccacgacggugucagccuucacgaacugcuugcggccgaacugaccaaggcccucaagaccaagcucgaucugucuagccucgccuacuccggaaaggacgccuga

SEQ ID NO: 4 - RNA, 633 nt, Artificial Sequence
  source: /note="Description of Artificial Sequence: Synthetic polynucleotide"
auguggaccuugggacggagagccguggcuggacuguuggccucuccuuccccggcacaagcccaaacucugacccgggucccuagaccggcagagcuggcuccccuguguggucggcggggacugagaacugauauugacgccacaugcacuccuaggcgcgcgagcuccaaucagcgcggccugaaccagaucuggaacgugaagaagcaguccgucuacuugaugaaccuccgcaaguccggcacucugggccauccgggaucccucgacgagacuaccuacgagcggcuggcggaagaaacccuggauucccuggccgaauucuucgaggaccuggccgacaagcccuacaccuuugaggacuacgacguguccuucggaucgggagugcugaccgugaagcucggcggagaucucgggacuuaugugaucaacaagcagacgccgaacaagcagaucuggcuuagcucacccucgagcggaccaaagcgcuacgacuggaccggcaaaaacuggguguacucccacgauggugucagccuucacgaacugcuggccgcggaacugaccaaggcccuuaagaccaagcucgaccucucaucccuggccuacuccgggaaagacgcguga

SEQ ID NO: 5 - protein, 210 aa, Homo sapiens
MWTLGRRAVAGLLASPSPAQAQTLTRVPRPAELAPLCGRRGLRTDIDATCTPRRASSNQRGLNQIWNVKKQSVYLMNLRKSGTLGHPGSLDETTYERLAEETLDSLAEFFEDLADKPYTFEDYDVSFGSGVLTVKLGGDLGTYVINKQTPNKQIWLSSPSSGPKRYDWTGKNWVYSHDGVSLHELLAAELTKALKTKLDLSSLAYSGKDA

SEQ ID NO: 6 - RNA, 140 nt, Artificial Sequence
  source: /note="Description of Artificial Sequence: Synthetic polynucleotide"
ggacagaucgccuggagacgccauccacgcuguuuugaccuccauagaagacaccgggaccgauccagccuccgcggccgggaacggugcauuggaacgcggauuccccgugccaagagugacucaccguccuugacacg

SEQ ID NO: 7 - RNA, 105 nt, Artificial Sequence
  source: /note="Description of Artificial Sequence: Synthetic polynucleotide"
cggguggcaucccugugaccccuccccagugccucuccuggcccuggaaguugccacuccagugcccaccagccuuguccuaauaaaauuaaguugcaucaagcu

SEQ ID NO: 8 - RNA, 105 nt, Artificial Sequence
  source: /note="Description of Artificial Sequence: Synthetic polynucleotide"
ggguggcaucccugugaccccuccccagugccucuccuggcccuggaaguugccacuccagugcccaccagccuuguccuaauaaaauuaaguugcaucaaagcu

SEQ ID NO: 9 - RNA, 878 nt, Artificial Sequence
  source: /note="Description of Artificial Sequence: Synthetic polynucleotide"
ggacagaucgccuggagacgccauccacgcuguuuugaccuccauagaagacaccgggaccgauccagccuccgcggccgggaacggugcauuggaacgcggauuccccgugccaagagugacucaccguccuugacacgauguggacccugggucggagagcuguggccggucugcuggcuucccccucaccggcacaagcgcagacccugacuagagugccuaggcccgcugaacucgcaccacugugcggcagacggggacuccggacugacaucgaugccaccuguaccccgcgaagggcaucuagcaaucagcgcggacugaaccagaucuggaacgugaagaagcaguccguguaccugaugaaucugcgcaaauccggcacucucggacacccgggaucgcuggaugagacuacuuacgagcgcuuggccgaagaaacccuggauucgcuggccgaguuuuucgaggaccuggccgacaagcccuacacguucgaggacuacgacguguccuucggaucgggcgugcugaccgugaagcucggcggggauuuggggaccuacgugaucaacaagcagacaccgaacaagcaaauuuggcucuccuccccuuccuccggaccuaagcgcuacgacuggaccgggaagaacugggucuacucccaugacggcgucagccuucacgaacugcuggccgccgaacugacuaaggcccucaaaacuaagcuggaccugucgagccuugccuauuccggaaaggacgccugacggguggcaucccugugaccccuccccagugccucuccuggcccuggaaguugccacuccagugcccaccagccuuguccuaauaaaauuaaguugcaucaagcu

SEQ ID NO: 10 - RNA, 878 nt, Artificial Sequence
  source: /note="Description of Artificial Sequence: Synthetic polynucleotide"
ggacagaucgccuggagacgccauccacgcuguuuugaccuccauagaagacaccgggaccgauccagccuccgcggccgggaacggugcauuggaacgcggauuccccgugccaagagugacucaccguccuugacacgauguggacccugggucggagagcuguggccggucugcuggcuucccccucaccggcacaagcgcagacccugacuagagugccuaggcccgcugaacucgcaccacugugcggcagacggggacuccggacugacaucgaugccaccuguaccccgcgaagggcaucuagcaaucagcgcggacugaaccagaucuggaacgugaagaagcaguccguguaccugaugaaucugcgcaaauccggcacucucggacacccgggaucgcuggaugagacuacuuacgagcgcuuggccgaagaaacccuggauucgcuggccgaguuuuucgaggaccuggccgacaagcccuacacguucgaggacuacgacguguccuucggaucgggcgugcugaccgugaagcucggcggggauuuggggaccuacgugaucaacaagcagacaccgaacaagcaaauuuggcucuccuccccuuccuccggaccuaagcgcuacgacuggaccgggaagaacugggucuacucccaugacggcgucagccuucacgaacugcuggccgccgaacugacuaaggcccucaaaacuaagcuggaccugucgagccuugccuauuccggaaaggacgccugaggguggcaucccugugaccccuccccagugccucuccuggcccuggaaguugccacuccagugcccaccagccuuguccuaauaaaauuaaguugcaucaaagcu

SEQ ID NO: 11 - RNA, 878 nt, Artificial Sequence
  source: /note="Description of Artificial Sequence: Synthetic polynucleotide"
ggacagaucgccuggagacgccauccacgcuguuuugaccuccauagaagacaccgggaccgauccagccuccgcggccgggaacggugcauuggaacgcggauuccccgugccaagagugacucaccguccuugacacgauguggacccugggacgcagagccguggcuggccuucuggccuccccaagcccugcccaagcccagaccuugacuagagugccuagaccggccgaacucgcuccccugugcggacggaggggacucaggacugacaucgacgcaacaugcacuccaagacgcgccuccagcaaccagcggggccucaaccagauuuggaacgugaaaaagcaguccgucuaucugaugaaccuccgcaaguccggcaccuuggggcaucccgggucacuggaugaaaccaccuacgaacggcuggccgaagagacucucgacucccuggccgaguucuucgaggaccuggcggauaagccguacacuuucgaggacuacgaugucucuuucggauccggcgugcugaccgugaagcucgguggcgaccucggaacuuacgugaucaacaagcaaacgcccaacaagcagaucuggcuguccucgccgucaucgggaccuaagcgcuacgauuggaccgggaagaauuggguguacucgcacgacggugucagccugcacgagcugcuugcggcggaacugaccaaggcacucaagaccaaacuggaccuguccagccuggccuacuccggaaaggacgccuagcggguggcaucccugugaccccuccccagugccucuccuggcccuggaaguugccacuccagugcccaccagccuuguccuaauaaaauuaaguugcaucaagcu

SEQ ID NO: 12 - RNA, 878 nt, Artificial Sequence
  source: /note="Description of Artificial Sequence: Synthetic polynucleotide"
ggacagaucgccuggagacgccauccacgcuguuuugaccuccauagaagacaccgggaccgauccagccuccgcggccgggaacggugcauuggaacgcggauuccccgugccaagagugacucaccguccuugacacgauguggacccugggacgcagagccguggcuggccuucuggccuccccaagcccugcccaagcccagaccuugacuagagugccuagaccggccgaacucgcuccccugugcggacggaggggacucaggacugacaucgacgcaacaugcacuccaagacgcgccuccagcaaccagcggggccucaaccagauuuggaacgugaaaaagcaguccgucuaucugaugaaccuccgcaaguccggcaccuuggggcaucccgggucacuggaugaaaccaccuacgaacggcuggccgaagagacucucgacucccuggccgaguucuucgaggaccuggcggauaagccguacacuuucgaggacuacgaugucucuuucggauccggcgugcugaccgugaagcucgguggcgaccucggaacuuacgugaucaacaagcaaacgcccaacaagcagaucuggcuguccucgccgucaucgggaccuaagcgcuacgauuggaccgggaagaauuggguguacucgcacgacggugucagccugcacgagcugcuugcggcggaacugaccaaggcacucaagaccaaacuggaccuguccagccuggccuacuccggaaaggacgccuagggguggcaucccugugaccccuccccagugccucuccuggcccuggaaguugccacuccagugcccaccagccuuguccuaauaaaauuaaguugcaucaaagcu

SEQ ID NO: 13 - RNA, 878 nt, Artificial Sequence
  source: /note="Description of Artificial Sequence: Synthetic polynucleotide"
ggacagaucgccuggagacgccauccacgcuguuuugaccuccauagaagacaccgggaccgauccagccuccgcggccgggaacggugcauuggaacgcggauuccccgugccaagagugacucaccguccuugacacgauguggacucugggccggagagcuguggcaggccuucucgccucgccauccccugcccaagcgcagacccugacuagggucccuaggccugccgaguuggcaccguugugcggucggagaggacugcgcaccgacaucgaugccaccuguacuccucggagagccucguccaaccagcggggccugaaccagaucuggaacgugaagaaacaguccgucuaccugaugaaccuccgcaagucgggaacccugggacauccggguucccuggaugagacuacguacgaacggcuggcggaagaaacccuggacucccuggcggaguucuucgaggaccuggcugacaagcccuacacuuuugaggacuacgacgugucauucggaagcggaguguugacagugaagcuggggggcgaucugggaaccuacgugaucaacaagcagaccccgaacaagcaaauuuggcuguccucacccuccuccggaccuaaacgcuacgacuggaccgggaagaacuggguguauagccacgacggugucagccuucacgaacugcuugcggccgaacugaccaaggcccucaagaccaagcucgaucugucuagccucgccuacuccggaaaggacgccugacggguggcaucccugugaccccuccccagugccucuccuggcccuggaaguugccacuccagugcccaccagccuuguccuaauaaaauuaaguugcaucaagcu

SEQ ID NO: 14 - RNA, 878 nt, Artificial Sequence
  source: /note="Description of Artificial Sequence: Synthetic polynucleotide"
ggacagaucgccuggagacgccauccacgcuguuuugaccuccauagaagacaccgggaccgauccagccuccgcggccgggaacggugcauuggaacgcggauuccccgugccaagagugacucaccguccuugacacgauguggacucugggccggagagcuguggcaggccuucucgccucgccauccccugcccaagcgcagacccugacuagggucccuaggccugccgaguuggcaccguugugcggucggagaggacugcgcaccgacaucgaugccaccuguacuccucggagagccucguccaaccagcggggccugaaccagaucuggaacgugaagaaacaguccgucuaccugaugaaccuccgcaagucgggaacccugggacauccggguucccuggaugagacuacguacgaacggcuggcggaagaaacccuggacucccuggcggaguucuucgaggaccuggcugacaagcccuacacuuuugaggacuacgacgugucauucggaagcggaguguugacagugaagcuggggggcgaucugggaaccuacgugaucaacaagcagaccccgaacaagcaaauuuggcuguccucacccuccuccggaccuaaacgcuacgacuggaccgggaagaacuggguguauagccacgacggugucagccuucacgaacugcuugcggccgaacugaccaaggcccucaagaccaagcucgaucugucuagccucgccuacuccggaaaggacgccugaggguggcaucccugugaccccuccccagugccucuccuggcccuggaaguugccacuccagugcccaccagccuuguccuaauaaaauuaaguugcaucaaagcu

SEQ ID NO: 15 - RNA, 878 nt, Artificial Sequence
  source: /note="Description of Artificial Sequence: Synthetic polynucleotide"
ggacagaucgccuggagacgccauccacgcuguuuugaccuccauagaagacaccgggaccgauccagccuccgcggccgggaacggugcauuggaacgcggauuccccgugccaagagugacucaccguccuugacacgauguggaccuugggacggagagccguggcuggacuguuggccucuccuuccccggcacaagcccaaacucugacccgggucccuagaccggcagagcuggcuccccuguguggucggcggggacugagaacugauauugacgccacaugcacuccuaggcgcgcgagcuccaaucagcgcggccugaaccagaucuggaacgugaagaagcaguccgucuacuugaugaaccuccgcaaguccggcacucugggccauccgggaucccucgacgagacuaccuacgagcggcuggcggaagaaacccuggauucccuggccgaauucuucgaggaccuggccgacaagcccuacaccuuugaggacuacgacguguccuucggaucgggagugcugaccgugaagcucggcggagaucucgggacuuaugugaucaacaagcagacgccgaacaagcagaucuggcuuagcucacccucgagcggaccaaagcgcuacgacuggaccggcaaaaacuggguguacucccacgauggugucagccuucacgaacugcuggccgcggaacugaccaaggcccuuaagaccaagcucgaccucucaucccuggccuacuccgggaaagacgcgugacggguggcaucccugugaccccuccccagugccucuccuggcccuggaaguugccacuccagugcccaccagccuuguccuaauaaaauuaaguugcaucaagcu

SEQ ID NO: 16 - RNA, 878 nt, Artificial Sequence
  source: /note="Description of Artificial Sequence: Synthetic polynucleotide"
ggacagaucgccuggagacgccauccacgcuguuuugaccuccauagaagacaccgggaccgauccagccuccgcggccgggaacggugcauuggaacgcggauuccccgugccaagagugacucaccguccuugacacgauguggaccuugggacggagagccguggcuggacuguuggccucuccuuccccggcacaagcccaaacucugacccgggucccuagaccggcagagcuggcuccccuguguggucggcggggacugagaacugauauugacgccacaugcacuccuaggcgcgcgagcuccaaucagcgcggccugaaccagaucuggaacgugaagaagcaguccgucuacuugaugaaccuccgcaaguccggcacucugggccauccgggaucccucgacgagacuaccuacgagcggcuggcggaagaaacccuggauucccuggccgaauucuucgaggaccuggccgacaagcccuacaccuuugaggacuacgacguguccuucggaucgggagugcugaccgugaagcucggcggagaucucgggacuuaugugaucaacaagcagacgccgaacaagcagaucuggcuuagcucacccucgagcggaccaaagcgcuacgacuggaccggcaaaaacuggguguacucccacgauggugucagccuucacgaacugcuggccgcggaacugaccaaggcccuuaagaccaagcucgaccucucaucccuggccuacuccgggaaagacgcgugaggguggcaucccugugaccccuccccagugccucuccuggcccuggaaguugccacuccagugcccaccagccuuguccuaauaaaauuaaguugcaucaaagcu